European Patent Application EP 4 528 274 A2, published March 26, 2025. Title: BIOMARKERS FOR NEUROPATHOLOGICAL CONDITIONS AND METHODS FOR DIAGNOSIS AND MONITORING THE EFFICACY OF TREATMENT. Applicant: Instituto de Medicina Molecular João Lobo Antunes. Application EP, filed November 5, 2024. The sequence listing filed with the application follows.

SEQUENCE LISTING (28 sequences)

SEQ ID NO: 1 - protein, 2463 aa, Homo sapiens
METSERPROTRPLEULYSTRPHISGLYPROALAMETALAARGLEUTRPGLYLEUCYSLEULEUVALLEUGLYPHETRPARGALASERLEUALACYSPROTHRSERCYSLYSCYSSERSERALAARGILETRPCYSTHRGLUPROSERPROGLYILEVALALAPHEPROARGLEUGLUPROASNSERVALASPPROGLUASNILETHRGLUILELEUILEALAASNGLNLYSARGLEUGLUILEILEASNGLUASPASPVALGLUALATYRVALGLYLEUARGASNLEUTHRILEVALASPSERGLYLEULYSPHEVALALATYRLYSALAPHELEULYSASNSERASNLEUARGHISILEASNPHETHRARGASNLYSLEUTHRSERLEUSERARGARGHISPHEARGHISLEUASPLEUSERASPLEUILELEUTHRGLYASNPROPHETHRCYSSERCYSASPILEMETTRPLEULYSTHRLEUGLNGLUTHRLYSSERSERPROASPTHRGLNASPLEUTYRCYSLEUASNGLUSERSERLYSASNMETPROLEUALAASNLEUGLNILEPROASNCYSGLYLEUPROSERALAARGLEUALAALAPROASNLEUTHRVALGLUGLUGLYLYSSERVALTHRLEUSERCYSSERVALGLYGLYASPPROLEUPROTHRLEUTYRTRPASPVALGLYASNLEUVALSERLYSHISMETASNGLUTHRSERHISTHRGLNGLYSERLEUARGILETHRASNILESERSERASPASPSERGLYLYSGLNILESERCYSVALALAGLUASNLEUVALGLYGLUASPGLNASPSERVALASNLEUTHRVALHISPHEALAPROTHRILETHRPHELEUGLUSERPROTHRSERASPHISHISTRPCYSILEPROPHETHRVALARGGLYASNPROLYSPROALALEUGLNTRPPHETYRASNGLYALAILELEUASNGLUSERLYSTYRILECYSTHRLYSILEHISVALTHRASNHISTHRGLUTYRHISGLYCYSLEUGLNLEUASPASNPROTHRHISMETASNASNGLYASPTYRTHRLEUMETALALYSASNGLUTYRGLYLYSASPGLUARGGLNILESERALAHISPHEMETGLYARGPROGLYVALASPTYRGLUTHRASNPROASNTYRPROGLUVALLEUTYRGLUASPTRPTHRTHRPROTHRASPILEGLYASPTHRTHRASNLYSSERASNGLUILEPROSERTHRASPVALALAASPGLNSERASNARGGLUHISLEUSERVALTYRALAVALVALVALILEALASERVALVALGLYPHECYSLEULEUVALMETLEULEULEULEULYSLEUALAARGHISSERLYSPHEGLYMETLYSGLYPROALASERVALILESERASNASPASPASPSERALASERPROLEUHISHISILESERASNGLYSERASNTHRPROSERSERSERGLUGLYGLYPROASPALAVALILEILEGLYMETTHRLYSILEPROVALILEGLUASNPROGLNTYRPHEGLYILETHRASNSERGLNLEULYSPROASPTHRPHEVALGLNHISILELYSARGHISASNILEVALLEULYSARGGLULEUGLYGLUGLYALAPHEGLYLYSVALPHELEUALAGLUCYSTYRASNLEUCYSPROGLUGLNASPLYSILELEUVALALAVALLYSTHRLEULYSASPALASERASPASNALAARGLYSASPPHEHISARGGLUALAGLULEULEUTHRASNLEUGLNHISGLUHISILEVALLYSPHETYRGLYVALCYSVALGLUGLYASPPROLEUILEMETVALPHEGLUTYRMETLYSHISGLYASPLEUASNLYSPHELEUARGALAHISGLYPROASPALAVALLEUMETALAGLUGLYASNPROPROTHRGLULEUTHRGLNSERGLNMETLEUHISILEALAGLNGLNILEALAALAGLYMETVALTYRLEUALASERGLNHISPHEVALHISARGASPLEUALATHRARGASNCYSLEUVALGLYGLUASNLEULEUVALLYSILEGLYASPPHEGLYMETSERARGASPVALTYRSERTHRASPTYRTYRARGVALGLYGLYHISTHRMETLEUPROILEARGTRPMETPROPROGLUSERILEMETTYRARGLYSPHETHRTHRGLUSERASPVALTRPSERLEUGLYVALVALLEUTRPGLUILEPHETHRTYRGLYLYSGLNPROTRPTYRGLNLEUSERASNASNGLUVALILEGLUCYSILETHRGLNGLYARGVALLEUGLNARGPROARGTHRCYSPROGLNGLUVALTYRGLULEUMETLEUGLYCYSTRPGLNARGGLUPROHISTHRARGLYSASNILELYSSERILEHISTHRLEULEUGLNASNLEUALALYSALASERPROVALTYRLEUASPILELEUGLY

SEQ ID NO: 2 - protein, 903 aa, Homo sapiens
SERGLNLEULYSPROASPTHRPHEVALGLNHISILELYSARGHISASNILEVALLEULYSARGGLULEUGLYGLUGLYALAPHEGLYLYSVALPHELEUALAGLUCYSTYRASNLEUCYSPROGLUGLNASPLYSILELEUVALALAVALLYSTHRLEULYSASPALASERASPASNALAARGLYSASPPHEHISARGGLUALAGLULEULEUTHRASNLEUGLNHISGLUHISILEVALLYSPHETYRGLYVALCYSVALGLUGLYASPPROLEUILEMETVALPHEGLUTYRMETLYSHISGLYASPLEUASNLYSPHELEUARGALAHISGLYPROASPALAVALLEUMETALAGLUGLYASNPROPROTHRGLULEUTHRGLNSERGLNMETLEUHISILEALAGLNGLNILEALAALAGLYMETVALTYRLEUALASERGLNHISPHEVALHISARGASPLEUALATHRARGASNCYSLEUVALGLYGLUASNLEULEUVALLYSILEGLYASPPHEGLYMETSERARGASPVALTYRSERTHRASPTYRTYRARGVALGLYGLYHISTHRMETLEUPROILEARGTRPMETPROPROGLUSERILEMETTYRARGLYSPHETHRTHRGLUSERASPVALTRPSERLEUGLYVALVALLEUTRPGLUILEPHETHRTYRGLYLYSGLNPROTRPTYRGLNLEUSERASNASNGLUVALILEGLUCYSILETHRGLNGLYARGVALLEUGLNARGPROARGTHRCYSPROGLNGLUVALTYRGLULEUMETLEUGLYCYSTRPGLNARGGLUPROHISTHRARGLYSASNILELYSSERILEHISTHRLEULEUGLNASNLEUALALYSALASERPROVALTYRLEUASPILELEUGLY

SEQ ID NO: 3 - protein, 1560 aa, Homo sapiens
METSERPROTRPLEULYSTRPHISGLYPROALAMETALAARGLEUTRPGLYLEUCYSLEULEUVALLEUGLYPHETRPARGALASERLEUALACYSPROTHRSERCYSLYSCYSSERSERALAARGILETRPCYSTHRGLUPROSERPROGLYILEVALALAPHEPROARGLEUGLUPROASNSERVALASPPROGLUASNILETHRGLUILELEUILEALAASNGLNLYSARGLEUGLUILEILEASNGLUASPASPVALGLUALATYRVALGLYLEUARGASNLEUTHRILEVALASPSERGLYLEULYSPHEVALALATYRLYSALAPHELEULYSASNSERASNLEUARGHISILEASNPHETHRARGASNLYSLEUTHRSERLEUSERARGARGHISPHEARGHISLEUASPLEUSERASPLEUILELEUTHRGLYASNPROPHETHRCYSSERCYSASPILEMETTRPLEULYSTHRLEUGLNGLUTHRLYSSERSERPROASPTHRGLNASPLEUTYRCYSLEUASNGLUSERSERLYSASNMETPROLEUALAASNLEUGLNILEPROASNCYSGLYLEUPROSERALAARGLEUALAALAPROASNLEUTHRVALGLUGLUGLYLYSSERVALTHRLEUSERCYSSERVALGLYGLYASPPROLEUPROTHRLEUTYRTRPASPVALGLYASNLEUVALSERLYSHISMETASNGLUTHRSERHISTHRGLNGLYSERLEUARGILETHRASNILESERSERASPASPSERGLYLYSGLNILESERCYSVALALAGLUASNLEUVALGLYGLUASPGLNASPSERVALASNLEUTHRVALHISPHEALAPROTHRILETHRPHELEUGLUSERPROTHRSERASPHISHISTRPCYSILEPROPHETHRVALARGGLYASNPROLYSPROALALEUGLNTRPPHETYRASNGLYALAILELEUASNGLUSERLYSTYRILECYSTHRLYSILEHISVALTHRASNHISTHRGLUTYRHISGLYCYSLEUGLNLEUASPASNPROTHRHISMETASNASNGLYASPTYRTHRLEUMETALALYSASNGLUTYRGLYLYSASPGLUARGGLNILESERALAHISPHEMETGLYARGPROGLYVALASPTYRGLUTHRASNPROASNTYRPROGLUVALLEUTYRGLUASPTRPTHRTHRPROTHRASPILEGLYASPTHRTHRASNLYSSERASNGLUILEPROSERTHRASPVALALAASPGLNSERASNARGGLUHISLEUSERVALTYRALAVALVALVALILEALASERVALVALGLYPHECYSLEULEUVALMETLEULEULEULEULYSLEUALAARGHISSERLYSPHEGLYMETLYSGLYPROALASERVALILESERASNASPASPASPSERALASERPROLEUHISHISILESERASNGLYSERASNTHRPROSERSERSERGLUGLYGLYPROASPALAVALILEILEGLYMETTHRLYSILEPROVALILEGLUASNPROGLNTYRPHEGLYILETHRASN

SEQ ID NO: 4 - protein, 12 aa, synthetic construct
GLYILETHRASN

SEQ ID NO: 5 - protein, 15 aa, synthetic construct
PHEGLYILETHRASN

SEQ ID NO: 6 - protein, 18 aa, synthetic construct
TYRPHEGLYILETHRASN

SEQ ID NO: 7 - protein, 21 aa, synthetic construct
GLNTYRPHEGLYILETHRASN

SEQ ID NO: 8 - protein, 24 aa, synthetic construct
PROGLNTYRPHEGLYILETHRASN

SEQ ID NO: 9 - protein, 27 aa, synthetic construct
ASNPROGLNTYRPHEGLYILETHRASN

SEQ ID NO: 10 - protein, 30 aa, synthetic construct
GLUASNPROGLNTYRPHEGLYILETHRASN

SEQ ID NO: 11 - protein, 12 aa, synthetic construct
SERGLNLEULYS

SEQ ID NO: 12 - protein, 15 aa, synthetic construct
SERGLNLEULYSPRO

SEQ ID NO: 13 - protein, 18 aa, synthetic construct
SERGLNLEULYSPROASP

SEQ ID NO: 14 - protein, 21 aa, synthetic construct
SERGLNLEULYSPROASPTHR

SEQ ID NO: 15 - protein, 24 aa, synthetic construct
SERGLNLEULYSPROASPTHRPHE

SEQ ID NO: 16 - protein, 27 aa, synthetic construct
SERGLNLEULYSPROASPTHRPHEVAL

SEQ ID NO: 17 - protein, 30 aa, synthetic construct
SERGLNLEULYSPROASPTHRPHEVALGLN

SEQ ID NO: 18 - protein, 30 aa, synthetic construct
PHEGLYILETHRASNSERGLNLEULYSPRO

SEQ ID NO: 19 - protein, 48 aa, synthetic construct
PROGLNTYRPHEGLYILETHRASNSERGLNLEULYSPROASPTHRPHE

SEQ ID NO: 20 - protein, 42 aa, synthetic construct
ILETHRASNSERGLNLEULYSPROASPTHRPHEVALGLNHIS

SEQ ID NO: 21 - protein, 33 aa, synthetic construct
TYRGLYARGLYSLYSARGARGGLNARGARGARG

SEQ ID NO: 22 - protein, 69 aa, synthetic construct
TYRGLYARGLYSLYSARGARGGLNARGARGARGLYSLYSPHEGLYILETHRASNSERGLNLEULYSPRO

SEQ ID NO: 23 - protein, 87 aa, synthetic construct
TYRGLYARGLYSLYSARGARGGLNARGARGARGLYSLYSPROGLNTYRPHEGLYILETHRASNSERGLNLEULYSPROASPTHRPHE

SEQ ID NO: 24 - protein, 81 aa, synthetic construct
TYRGLYARGLYSLYSARGARGGLNARGARGARGLYSLYSILETHRASNSERGLNLEULYSPROASPTHRPHEVALGLNHIS

SEQ ID NO: 25 - protein, 81 aa, synthetic construct
TYRGLYARGLYSLYSARGARGGLNARGARGARGPROGLNTYRPHEGLYILETHRASNSERGLNLEULYSPROASPTHRPHE

SEQ ID NO: 26 - protein, 69 aa, synthetic construct
TYRGLYARGLYSLYSARGARGGLNARGARGARGPROPROPHEGLYILETHRASNSERGLNLEULYSPRO

SEQ ID NO: 27 - protein, 66 aa, synthetic construct
TYRGLYARGLYSLYSARGARGGLNARGARGARGGLNPHEGLYILETHRASNSERGLNLEULYSPRO

SEQ ID NO: 28 - protein, 66 aa, synthetic construct
TYRGLYARGLYSLYSARGARGGLNARGARGARGGLUPHEGLYILETHRASNSERGLNLEULYSPRO